European Patent Application EP 4 202 044 A2, published June 28, 2023. Title: POLYPEPTIDE HAVING CEPHALOSPORIN C ACYLASE ACTIVITY AND USE THEREOF. Applicant: AMICOGEN, INC. The sequence listing filed with the application follows.

SEQUENCE LISTING (32 sequences)

SEQ ID NO: 1 - protein, 692 aa, synthetic construct
  REGION 1..692: note = Protein (692 aa) of wild-type Gl-7-ACA acylase from Pseudomonassp. GK16, comprising alpha- and beta-subunits and a spacer therebetween
MEPTSTPQAPIAAYKPRSNEILWDGYGVPHIYGVDAPSAFYGYGWAQARSHGDNILRLYGEARGKGAEYWGPDYEQTTVWLLTNGVPERAQQWYAQQSPDFRANLDAFAAGINAYAQQNPDDISPEVRQVLPVSGADVVAHAHRLMNFLYVASPGRTLGEGDPPDLADQGSNSWAVAPGKTANGNALLLQNPHLSWTTDYFTYYEAHLVTPDFEIYGATQIGLPVIRFAFNQRMGITNTVNGMVGATNYRLTLQDGGYLYDGQVRPFERRQASYRLRQADGTTVDKPLEIRSSVHGPVFERADGTAVAVRVAGLDRPGMLEQYFDMITADSFDDYEAALARMQVPTFNIVYADREGTINYSFNGVAPKRAEGDIAFWQGLVPGDSSRYLWTETHPLDDLPRVTNPPGGFVQNSNDPPWTPTWPVTYTPKDFPSYLAPQTPHSLRAQQSVRLMSENDDLTLERFMALQLSHRAVMADRTLPDLIPAALIDPDPEVQAAARLLAAWDREFTSDSRAALLFEEWARLFAGQNFAGQAGFATPWSLDKPVSTPYGVRDPKAAVDQLRTAIANTKRKYGAIDRPFGDASRMILNDVNVPGAAGYGNLGSFRVFTWSDPDENGVRTPVHGETWVAMIEFSTPVRAYGLMSYGNSRQPGTTHYSDQIERVSRADFRELLLRREQVEAAVQERTPFNFKP

SEQ ID NO: 2 - protein, 2079 aa, synthetic construct
  REGION 1..2079: note = Gene (2079 bp) encoding the proten of SEQ ID NO: 1
ATGGAACCGACCAGCACCCCGCAGGCTCCGATCGCTGCTTATAAACCGCGTAGCAACGAAATCCTGTGGGATGGTTATGGTGTTCCGCATATCTATGGTGTTGACGCTCCGAGCGCTTTTTATGGTTATGGCTGGGCTCAGGCTCGTAGCCATGGTGATAACATCCTGCGTCTGTATGGTGAAGCTCGTGGTAAAGGCGCTGAATATTGGGGTCCGGATTACGAACAGACGACCGTTTGGCTGCTGACCAACGGTGTTCCGGAACGTGCTCAGCAGTGGTATGCTCAGCAGAGCCCGGATTTTCGTGCTAACCTGGATGCTTTTGCTGCTGGTATCAACGCTTATGCTCAGCAGAACCCGGATGATATCAGCCCGGAAGTTCGTCAGGTTCTGCCGGTTAGCGGTGCTGATGTTGTTGCTCATGCTCATCGTCTGATGAACTTTCTGTATGTTGCTAGCCCGGGTCGTACCCTGGGTGAAGGTGATCCGCCGGATCTGGCTGATCAGGGTAGCAACAGCTGGGCTGTTGCTCCGGGTAAAACCGCTAACGGTAACGCTCTGCTGCTGCAGAACCCTCATCTGAGCTGGACCACCGATTATTTTACCTATTATGAAGCTCATCTGGTTACCCCGGATTTTGAAATCTATGGTGCTACCCAGATCGGTCTGCCGGTTATCCGTTTTGCTTTTAACCAGCGTATGGGTATCACCAACACCGTTAACGGTATGGTTGGTGCTACCAACTATCGTCTGACCCTGCAGGATGGTGGTTATCTGTATGATGGTCAGGTTCGTCCGTTTGAACGTCGTCAGGCTAGCTATCGTCTGCGTCAGGCTGATGGTACCACCGTTGATAAACCGCTGGAAATCCGTTCCAGCGTTCATGGTCCGGTTTTTGAACGTGCTGATGGTACCGCTGTTGCTGTTCGTGTTGCTGGTCTGGATCGTCCGGGTATGCTGGAACAGTATTTTGATATGATCACCGCTGATAGCTTTGATGATTATGAAGCTGCTCTGGCTCGTATGCAGGTTCCGACCTTTAACATCGTTTATGCTGATCGTGAAGGTACCATCAACTATAGCTTTAACGGTGTTGCTCCGAAACGTGCTGAAGGTGACATCGCTTTTTGGCAGGGTCTGGTTCCGGGTGATAGCAGCCGTTATCTGTGGACCGAAACCCATCCGCTGGATGATCTGCCGCGTGTTACCAACCCGCCGGGTGGTTTTGTTCAGAACAGCAACGATCCGCCGTGGACCCCGACCTGGCCGGTTACCTATACCCCGAAAGATTTTCCGAGCTATCTGGCTCCGCAGACCCCGCATAGCCTGCGTGCTCAGCAGAGCGTTCGTCTGATGAGCGAAAACGATGATCTGACCCTGGAACGTTTTATGGCTCTGCAGCTGAGCCATCGTGCTGTTATGGCTGATCGTACCCTGCCGGATCTGATCCCGGCTGCTCTGATCGATCCGGATCCGGAAGTTCAGGCTGCTGCTCGTCTGCTGGCTGCGTGGGATCGTGAATTTACCAGCGATAGCCGTGCTGCTCTGCTGTTTGAAGAATGGGCTCGTCTGTTTGCTGGTCAGAACTTTGCTGGTCAGGCTGGCTTTGCTACCCCGTGGAGCCTGGATAAACCGGTTAGCACCCCGTATGGTGTTCGTGATCCGAAAGCTGCTGTTGATCAGCTGCGTACCGCTATCGCTAACACCAAACGTAAATATGGTGCTATCGATCGTCCGTTTGGTGATGCTAGCCGTATGATCCTGAACGATGTTAACGTTCCGGGTGCTGCTGGTTATGGTAACCTGGGTAGCTTTCGTGTTTTTACCTGGAGCGATCCGGATGAAAACGGTGTGCGTACCCCGGTTCATGGTGAAACCTGGGTTGCTATGATCGAATTTAGCACCCCGGTTCGTGCTTATGGTCTGATGAGCTATGGTAACAGCCGTCAGCCGGGTACCACCCATTATAGCGATCAGATCGAACGTGTTAGCCGTGCTGATTTTCGTGAACTGCTGCTGCGTCGTGAACAGGTTGAAGCTGCTGTTCAGGAACGTACCCCGTTTAACTTTAAACCGTGA

SEQ ID NO: 3 - protein, 158 aa, synthetic construct
  REGION 1..158: note = Alpha-subunit (158 aa) of wild-type Gl-7-ACA acylase proteinfrom Pseudomonas sp. GK16
EPTSTPQAPIAAYKPRSNEILWDGYGVPHIYGVDAPSAFYGYGWAQARSHGDNILRLYGEARGKGAEYWGPDYEQTTVWLLTNGVPERAQQWYAQQSPDFRANLDAFAAGINAYAQQNPDDISPEVRQVLPVSGADVVAHAHRLMNFLYVASPGRTLG

SEQ ID NO: 4 - protein, 522 aa, synthetic construct
  REGION 1..522: note = Beta-subunit (522 aa) of wild-type Gl-7-ACA acylase protein
SNSWAVAPGKTANGNALLLQNPHLSWTTDYFTYYEAHLVTPDFEIYGATQIGLPVIRFAFNQRMGITNTVNGMVGATNYRLTLQDGGYLYDGQVRPFERRQASYRLRQADGTTVDKPLEIRSSVHGPVFERADGTAVAVRVAGLDRPGMLEQYFDMITADSFDDYEAALARMQVPTFNIVYADREGTINYSFNGVAPKRAEGDIAFWQGLVPGDSSRYLWTETHPLDDLPRVTNPPGGFVQNSNDPPWTPTWPVTYTPKDFPSYLAPQTPHSLRAQQSVRLMSENDDLTLERFMALQLSHRAVMADRTLPDLIPAALIDPDPEVQAAARLLAAWDREFTSDSRAALLFEEWARLFAGQNFAGQAGFATPWSLDKPVSTPYGVRDPKAAVDQLRTAIANTKRKYGAIDRPFGDASRMILNDVNVPGAAGYGNLGSFRVFTWSDPDENGVRTPVHGETWVAMIEFSTPVRAYGLMSYGNSRQPGTTHYSDQIERVSRADFRELLLRREQVEAAVQERTPFNFKP

SEQ ID NO: 5 - protein, 11 aa, synthetic construct
  REGION 1..11: note = Spacer (11 aa)
EGDPPDLADQG

SEQ ID NO: 6 - protein, 692 aa, synthetic construct
  REGION 1..692: note = PM2 mutant (692 aa) comprising wild-type alpha-subunit ofGl-7-ACA asylase from GK16, and mutant beta-subunit, and aspacer therebetween
MEPTSTPQAPIAAYKPRSNEILWDGYGVPHIYGVDAPSAFYGYGWAQARSHGDNILRLYGEARGKGAEYWGPDYEQTTVWLLTNGVPERAQQWYAQQSPDFRANLDAFAAGINAYAQQNPDDISPEVRQVLPVSGADVVAHAHRLMNFLYVASPGRTLGEGDPPDLADQGSNSWAVAPGKTANGNALLLQNPHLSWTTDYFTYYEAHLVTPDFEVYGATQIGLPVIRVAFNQRMGITNTVNGMVGATNYRLTLQDGGYLYDGQVRPFERRQASYRLRQADGTTVDKPLEIRSSVHGPVFERADGTAVAVRVAGLDRPGMLEQTFDMITADSFDDYEAALARMQVPTLNIVYADREGTINYSFNGVAPKRAEGDIAFWQGLVPGDSSRYLWTETHPLDDLPRVTNPPGGFVQNSNDPPWTPTWPVTYTPKDFPSYLAPQTPHSLRAQQSVRLMSENDDLTLERFMALQLSHRAVMADRTLPDLIPAALIDPDPEVQAAARLLAAWDREFTSDSRAALLFEEWARLFAGQNFAGQAGFATPWSLDKPVSTPYGLRDPKAAVDQLRTAIANTKRKYGAIDRPFGDASRMILNDVNVPGAAGYGNLGSFRVFTWSDPDENGVRTPVHGETWVAMIEFSTPVRAYGLMSYGNSRQPGTTHYSDQIERVSRADFRELLLRREQVEAAVQERTPFNFKP

SEQ ID NO: 7 - protein, 2079 aa, synthetic construct
  REGION 1..2079: note = Gene (2079 bp) encoding PM2 mutant
ATGGAACCGACCAGCACCCCGCAGGCTCCGATCGCTGCTTATAAACCGCGTAGCAACGAAATCCTGTGGGATGGTTATGGTGTTCCGCATATCTATGGTGTTGACGCTCCGAGCGCTTTTTATGGTTATGGCTGGGCTCAGGCTCGTAGCCATGGTGATAACATCCTGCGTCTGTATGGTGAAGCTCGTGGTAAAGGCGCTGAATATTGGGGTCCGGATTACGAACAGACGACCGTTTGGCTGCTGACCAACGGTGTTCCGGAACGTGCTCAGCAGTGGTATGCTCAGCAGAGCCCGGATTTTCGTGCTAACCTGGATGCTTTTGCTGCTGGTATCAACGCTTATGCTCAGCAGAACCCGGATGATATCAGCCCGGAAGTTCGTCAGGTTCTGCCGGTTAGCGGTGCTGATGTTGTTGCTCATGCTCATCGTCTGATGAACTTTCTGTATGTTGCTAGCCCGGGTCGTACCCTGGGTGAAGGTGATCCGCCGGATCTGGCTGATCAGGGTAGCAACAGCTGGGCTGTTGCTCCGGGTAAAACCGCTAACGGTAACGCTCTGCTGCTGCAGAACCCTCATCTGAGCTGGACCACCGATTATTTTACCTATTATGAAGCTCATCTGGTTACCCCGGATTTTGAAGTGTATGGTGCTACCCAGATCGGTCTGCCGGTTATCCGTGTTGCTTTTAACCAGCGTATGGGTATCACCAACACCGTTAACGGTATGGTTGGTGCTACCAACTATCGTCTGACCCTGCAGGATGGTGGTTATCTGTATGATGGTCAGGTTCGTCCGTTTGAACGTCGTCAGGCTAGCTATCGTCTGCGTCAGGCTGATGGTACCACCGTTGATAAACCGCTGGAAATCCGTTCCAGCGTTCATGGTCCGGTTTTTGAACGTGCTGATGGTACCGCTGTTGCTGTTCGTGTTGCTGGTCTGGATCGTCCGGGTATGCTGGAACAGACTTTTGATATGATCACCGCTGATAGCTTTGATGATTATGAAGCTGCTCTGGCTCGTATGCAGGTTCCGACCTTGAACATCGTTTATGCTGATCGTGAAGGTACCATCAACTATAGCTTTAACGGTGTTGCTCCGAAACGTGCTGAAGGTGACATCGCTTTTTGGCAGGGTCTGGTTCCGGGTGATAGCAGCCGTTATCTGTGGACCGAAACCCATCCGCTGGATGATCTGCCGCGTGTTACCAACCCGCCGGGTGGTTTTGTTCAGAACAGCAACGATCCGCCGTGGACCCCGACCTGGCCGGTTACCTATACCCCGAAAGATTTTCCGAGCTATCTGGCTCCGCAGACCCCGCATAGCCTGCGTGCTCAGCAGAGCGTTCGTCTGATGAGCGAAAACGATGATCTGACCCTGGAACGTTTTATGGCTCTGCAGCTGAGCCATCGTGCTGTTATGGCTGATCGTACCCTGCCGGATCTGATCCCGGCTGCTCTGATCGATCCGGATCCGGAAGTTCAGGCTGCTGCTCGTCTGCTGGCTGCGTGGGATCGTGAATTTACCAGCGATAGCCGTGCTGCTCTGCTGTTTGAAGAATGGGCTCGTCTGTTTGCTGGTCAGAACTTTGCTGGTCAGGCTGGCTTTGCTACCCCGTGGAGCCTGGATAAACCGGTTAGCACCCCGTATGGTCTGCGTGATCCGAAAGCTGCTGTTGATCAGCTGCGTACCGCTATCGCTAACACCAAACGTAAATATGGTGCTATCGATCGTCCGTTTGGTGATGCTAGCCGTATGATCCTGAACGATGTTAACGTTCCGGGTGCTGCTGGTTATGGTAACCTGGGTAGCTTTCGTGTTTTTACCTGGAGCGATCCGGATGAAAACGGTGTGCGTACCCCGGTTCATGGTGAAACCTGGGTTGCTATGATCGAATTTAGCACCCCGGTTCGTGCTTATGGTCTGATGAGCTATGGTAACAGCCGTCAGCCGGGTACCACCCATTATAGCGATCAGATCGAACGTGTTAGCCGTGCTGATTTTCGTGAACTGCTGCTGCGTCGTGAACAGGTTGAAGCTGCTGTTCAGGAACGTACCCCGTTTAACTTTAAACCGTGA

SEQ ID NO: 8 - protein, 522 aa, synthetic construct
  REGION 1..522: note = Beta-subunit of mutant PM2 protein
SNSWAVAPGKTANGNALLLQNPHLSWTTDYFTYYEAHLVTPDFEVYGATQIGLPVIRVAFNQRMGITNTVNGMVGATNYRLTLQDGGYLYDGQVRPFERRQASYRLRQADGTTVDKPLEIRSSVHGPVFERADGTAVAVRVAGLDRPGMLEQTFDMITADSFDDYEAALARMQVPTLNIVYADREGTINYSFNGVAPKRAEGDIAFWQGLVPGDSSRYLWTETHPLDDLPRVTNPPGGFVQNSNDPPWTPTWPVTYTPKDFPSYLAPQTPHSLRAQQSVRLMSENDDLTLERFMALQLSHRAVMADRTLPDLIPAALIDPDPEVQAAARLLAAWDREFTSDSRAALLFEEWARLFAGQNFAGQAGFATPWSLDKPVSTPYGLRDPKAAVDQLRTAIANTKRKYGAIDRPFGDASRMILNDVNVPGAAGYGNLGSFRVFTWSDPDENGVRTPVHGETWVAMIEFSTPVRAYGLMSYGNSRQPGTTHYSDQIERVSRADFRELLLRREQVEAAVQERTPFNFKP

SEQ ID NO: 9 - protein, 692 aa, synthetic construct
  REGION 1..692: note = mutant CSH17 protein
MEPTSTPQAPINAYKPRSNEILWDDYGVPHIYGVDAPSAFYGYGWAQARSHGDNILRLYGEARGKGAEYWGPDYEQTTVWLLTNGVPERAQQWYAQQSPDFRANLDAFAAGINAYAQQNPDDISPEVRQVLPVSGADVVAHAHRLMNFLYVASPGRTLGEGDPPDLADQGSNSWAVAPGKTANGNALLLQNPHLSWTTDYFTYYEAHLVTPDFEVYGATQIGLPVIRVAFNQRMGITNTVNGMVGATNYRLTLQDGGYLYDGQVRPFERRQASYRLRQADGTTVDKPLEIRSSVHGPVFERADGTTVAVRVAGLDRPGMLEQTFDMITADSFDDYEAALARMQVPTLNYVYADREGTINYSFNGVAPKRAEGDIAFWQGLVPGDSSRYLWTETHPLDDLPRVTNPPGGFVQNSNDPPWTPTWPVTYTPKDFPSYLAPQTPHSLRAQQSVRLMSENDDLTLERFMALQLSHRAVMADRTLPDLIPAALIDPDPEVQAAARLLAAWDREFTSDSRAALLFEEWARLFAGQNFAGQAGFATPWSLDKPVSTPYGLRDPKAAVDQLRTAIANTKRKYGAIDRPFGDASRMILNDVNVPGAAGYGNLGSFRVFTWSDPDENGVRTPVHGETWVAMIEFSTPVRAYGLMSYGNSRQPGTTHYSDQIERVSRADFRELLLRREQVEAAVQERTPFNFKP

SEQ ID NO: 10 - protein, 158 aa, synthetic construct
  REGION 1..158: note = Alpha-subunit of mutant CSH17 protein
EPTSTPQAPINAYKPRSNEILWDDYGVPHIYGVDAPSAFYGYGWAQARSHGDNILRLYGEARGKGAEYWGPDYEQTTVWLLTNGVPERAQQWYAQQSPDFRANLDAFAAGINAYAQQNPDDISPEVRQVLPVSGADVVAHAHRLMNFLYVASPGRTLG

SEQ ID NO: 11 - protein, 522 aa, synthetic construct
  REGION 1..522: note = Beta-subunit of mutant CSH17 protein
SNSWAVAPGKTANGNALLLQNPHLSWTTDYFTYYEAHLVTPDFEVYGATQIGLPVIRVAFNQRMGITNTVNGMVGATNYRLTLQDGGYLYDGQVRPFERRQASYRLRQADGTTVDKPLEIRSSVHGPVFERADGTTVAVRVAGLDRPGMLEQTFDMITADSFDDYEAALARMQVPTLNYVYADREGTINYSFNGVAPKRAEGDIAFWQGLVPGDSSRYLWTETHPLDDLPRVTNPPGGFVQNSNDPPWTPTWPVTYTPKDFPSYLAPQTPHSLRAQQSVRLMSENDDLTLERFMALQLSHRAVMADRTLPDLIPAALIDPDPEVQAAARLLAAWDREFTSDSRAALLFEEWARLFAGQNFAGQAGFATPWSLDKPVSTPYGLRDPKAAVDQLRTAIANTKRKYGAIDRPFGDASRMILNDVNVPGAAGYGNLGSFRVFTWSDPDENGVRTPVHGETWVAMIEFSTPVRAYGLMSYGNSRQPGTTHYSDQIERVSRADFRELLLRREQVEAAVQERTPFNFKP

SEQ ID NO: 12 - protein, 692 aa, synthetic construct
  REGION 1..692: note = mutant TEP11 protein
MEPTSTPQAPINAYKPRSNEILWDDYGVPHIYGVDAPSAFYGYGWAQARSHGDNILRLYGEARGKGAEYWGPDYEQTTVWLLTNGVPERAQQWYAQQSPDFRANLDAFAAGINAYAQQNPDDISPEVRQVLPVSGADVVAHAHRLMNFLYVASPGRTLGEGDPPDLADQGSNSWAVAPGKTANGNALLLQNPHLSWTTDYFTYYEAHLVTPDFEVYGATQIGLPVIRVAFNQRMGITNTVNGMVGATNYRLTLQDGGYLYDGQVRPFERRQASYRLRQADGTTVDKPLEIRSSVHGPVFERADGTTVAVRVAGLDRPGMLEQTFDMITADSFDDYEAALARMQVPTLNYVYADREGTINYSFNGVAPKRAEGDIAFWQGLVPGDSSRYLWTETHPLDDLPRVTNPPGGFVQNSNDPPWTPTWPVTYTPKDFPSYLAPQTPHSLRAQQSVRLMSENDDLTLERFMALQLSHRAVMADRTLPDLIPAALIDPDPEVQAAARLLAAWDREFTSDSRAALLFEEWARLFAGQNFAGQAGFATPWSLDKPVSTPYGLRDPKAAVDQLRTAIANTKRKYGAIDRPFGDASRMILNDVNVPGAAGYGNLGSFRVFTWSDPDENGVRTPVTGETWVAMIEFSTPVRAYGLMSYGNSRQPGTTHYSDQIERVSRADFRELLLRREQVEAAVQERTPFNFKP

SEQ ID NO: 13 - protein, 158 aa, synthetic construct; identical to SEQ ID NO: 10
  REGION 1..158: note = Alpha-subunit of mutant TEP11 protein

SEQ ID NO: 14 - protein, 522 aa, synthetic construct
  REGION 1..522: note = Beta-subunit of mutant TEP11
SNSWAVAPGKTANGNALLLQNPHLSWTTDYFTYYEAHLVTPDFEVYGATQIGLPVIRVAFNQRMGITNTVNGMVGATNYRLTLQDGGYLYDGQVRPFERRQASYRLRQADGTTVDKPLEIRSSVHGPVFERADGTTVAVRVAGLDRPGMLEQTFDMITADSFDDYEAALARMQVPTLNYVYADREGTINYSFNGVAPKRAEGDIAFWQGLVPGDSSRYLWTETHPLDDLPRVTNPPGGFVQNSNDPPWTPTWPVTYTPKDFPSYLAPQTPHSLRAQQSVRLMSENDDLTLERFMALQLSHRAVMADRTLPDLIPAALIDPDPEVQAAARLLAAWDREFTSDSRAALLFEEWARLFAGQNFAGQAGFATPWSLDKPVSTPYGLRDPKAAVDQLRTAIANTKRKYGAIDRPFGDASRMILNDVNVPGAAGYGNLGSFRVFTWSDPDENGVRTPVTGETWVAMIEFSTPVRAYGLMSYGNSRQPGTTHYSDQIERVSRADFRELLLRREQVEAAVQERTPFNFKP

SEQ ID NO: 15 - DNA, 20 bp, synthetic construct
  misc_feature 1..20: note = T3 primer
  source 1..20: mol_type = other DNA
aattaaccctcactaaaggg

SEQ ID NO: 16 - DNA, 20 bp, synthetic construct
  misc_feature 1..20: note = T7 primer
  source 1..20: mol_type = other DNA
taatacgactcactataggg

SEQ ID NO: 17 - DNA, 20 bp, synthetic construct
  misc_feature 1..20: note = M13-F primer
  source 1..20: mol_type = other DNA
ttgtaaaacgacggccagtg

SEQ ID NO: 18 - DNA, 19 bp, synthetic construct
  misc_feature 1..19: note = M13-R primer
  source 1..19: mol_type = other DNA
ggaaacagctatgaccatg

SEQ ID NO: 19 - DNA, 30 bp, synthetic construct
  misc_feature 1..30: note = SH24a-F primer (non-opti)
  source 1..30: mol_type = other DNA
gaaatcctgtgggatgrytatggtgttccg

SEQ ID NO: 20 - DNA, 30 bp, synthetic construct
  misc_feature 1..30: note = SH24a-R primer
  source 1..30: mol_type = other DNA
cggaacaccatarycatcccacaggatttc

SEQ ID NO: 21 - DNA, 33 bp, synthetic construct
  misc_feature 1..33: note = SH179b-F primer
  source 1..33: mol_type = other DNA
gttccgacccttaacwwygtttatgctgatcgt

SEQ ID NO: 22 - DNA, 33 bp, synthetic construct
  misc_feature 1..33: note = SH179b-R primer
  source 1..33: mol_type = other DNA
acgatcagcataaacrwwgttaagggtcggaac

SEQ ID NO: 23 - DNA, 34 bp, synthetic construct
  misc_feature 1..34: note = SM7_F priemr
  source 1..34: mol_type = other DNA
gttccgacctttaactatgtttatgctgatcgtg

SEQ ID NO: 24 - DNA, 34 bp, synthetic construct
  misc_feature 1..34: note = SM7_R priemr
  source 1..34: mol_type = other DNA
cacgatcagcataaacatagttaaaggtcggaac

SEQ ID NO: 25 - DNA, 36 bp, synthetic construct
  misc_feature 1..36: note = SM10_F priemr
  source 1..36: mol_type = other DNA
gaaatcctgtgggatgactatggtgttccgcatatc

SEQ ID NO: 26 - DNA, 36 bp, synthetic construct
  misc_feature 1..36: note = SM10_R priemr
  source 1..36: mol_type = other DNA
gatatgcggaacaccatagtcatcccacaggatttc

SEQ ID NO: 27 - DNA, 34 bp, synthetic construct
  misc_feature 1..34: note = SM25_F priemr
  source 1..34: mol_type = other DNA
cgtgctgatggtaccaccgttgctgttcgtgttg

SEQ ID NO: 28 - DNA, 34 bp, synthetic construct
  misc_feature 1..34: note = SM25_R priemr
  source 1..34: mol_type = other DNA
caacacgaacagcaacggtggtaccatcagcacg

SEQ ID NO: 29 - DNA, 36 bp, synthetic construct
  misc_feature 1..36: note = SM43_F priemr
  source 1..36: mol_type = other DNA
ccgcaggctccgatcaatgcttataaaccgcgtagc

SEQ ID NO: 30 - DNA, 36 bp, synthetic construct
  misc_feature 1..36: note = SM43_R priemr
  source 1..36: mol_type = other DNA
gctacgcggtttataagcattgatcggagcctgcgg

SEQ ID NO: 31 - DNA, 35 bp, synthetic construct
  misc_feature 1..35: note = SM52_F priemr
  source 1..35: mol_type = other DNA
gtgcgtaccccggttacgggtgaaacctgggttgc

SEQ ID NO: 32 - DNA, 35 bp, synthetic construct
  misc_feature 1..35: note = SM52_R priemr
  source 1..35: mol_type = other DNA
gcaacccaggtttcacccgtaaccggggtacgcac